European Patent Application EP 4 803 625 A1, published September 9, 2026. Title: 一种构建用于异种输血的基因工程动物的方法. Applicant: 成都中科奥格生物科技有限公司. The sequence listing filed with the application follows.

SEQUENCE LISTING (11 sequences)

SEQ ID NO: 1 - RNA, 21 nt, synthetic construct
  source 1..21: mol_type = other RNA
gaaggccgcacccttctccgc

SEQ ID NO: 2 - RNA, 21 nt, synthetic construct
  source 1..21: mol_type = other RNA
gtctgctgcctccttttccta

SEQ ID NO: 3 - RNA, 21 nt, synthetic construct
  source 1..21: mol_type = other RNA
ggctccttctcgattatgggc

SEQ ID NO: 4 - RNA, 21 nt, synthetic construct
  source 1..21: mol_type = other RNA
gccctggcttaacctgattct

SEQ ID NO: 5 - RNA, 21 nt, synthetic construct
  source 1..21: mol_type = other RNA
gattcttgggcgttgtcctgc

SEQ ID NO: 6 - DNA, 5028 bp, synthetic construct
  source 1..5028: mol_type = other DNA
gtcactgattggccgcttctcctcccgccgtgtgtgaaaacacaaatggcgtgttttggttggagtaaagctcctgtcagttacagcctcgggagtgcgcagcctcccaggaactctcgcattgccccctgggtgggtaggtaggtggggtggagagagctgcacaggcgggcgctgtcggcctcctgcggggggaggggagggtcagtgaaagtggctcccgcgcgggcgtcctgccaccctcccctccgggggagtcggtttacccgccgcctgctcggctttggtatctgattggctgctgaagtcctgggaacggccccttgttattggcttgggtcccaaatgagcgaaaccactacgcgagtcggcagggaggcggtctttggtacggccctccccgaggccagcgccgcagtgtctggcccctcgcccctgcgcaacgtggcaggaagcgcgcgcaggaggcgggggcgggctgccgggccgaggcttctgggtggtggtgactgcggctccgccctgggcgtccgccgcctgaaggacgagactagctctctacctgctctcggacccgtgggggtggggggtggaggaaggagtggggggtcggtcctgctggcttgtgggtgggaggcgcatgttctccaaaaacccgcgcgagctgcaatcctgagggagctgcagtggaggaggcggagagaaggccgcacccttctccgcagggggaggggagtgccgcaatacctttatgggagttctctgctgcctccttttcctaaggaccgccctgggcctagaaaaatccctccctcccccgcgatctcgtcatcgcctccatgtcagtttggctccggtgcccgtcagtgggcagagcgcacatcgcccacagtccccgagaagttggggggaggggtcggcaattgaaccggtgcctagagaaggtggcgcggggtaaactgggaaagtgatgtcgtgtactggctccgcctttttcccgagggtgggggagaaccgtatataagtgcagtagtcgccgtgaacgttctttttcgcaacgggtttgccgccagaacacaggtaagtgccgtgtgtggttcccgcgggcctggcctctttacgggttatggcccttgcgtgccttgaattacttccacgcccctggctgcagtacgtgattcttgatcccgagcttcgggttggaagtgggtgggagagttcgaggccttgcgcttaaggagccccttcgcctcgtgcttgagttgaggcctggcttgggcgctggggccgccgcgtgcgaatctggtggcaccttcgcgcctgtctcgctgctttcgataagtctctagccatttaaaatttttgatgacctgctgcgacgctttttttctggcaagatagtcttgtaaatgcgggccaagatctgcacactggtatttcggtttttggggccgcgggcggcgacggggcccgtgcgtcccagcgcacatgttcggcgaggcggggcctgcgagcgcggccaccgagaatcggacgggggtagtctcaagctggccggcctgctctggtgcctggcctcgcgccgccgtgtatcgccccgccctgggcggcaaggctggcccggtcggcaccagttgcgtgagcggaaagatggccgcttcccggccctgctgcagggagctcaaaatggaggacgcggcgctcgggagagcgggcgggtgagtcacccacacaaaggaaaagggcctttccgtcctcagccgtcgcttcatgtgactccacggagtaccgggcgccgtccaggcacctcgattagttctcgagcttttggagtacgtcgtctttaggttggggggaggggttttatgcgatggagtttccccacactgagtgggtggagactgaagttaggccagcttggcacttgatgtaattctccttggaatttgccctttttgagtttggatcttggttcattctcaagcctcagacagtggttcaaagtttttttcttccatttcaggtgtcgtgaggatctatttccggtgaattcctcgagactagttctagagcccaccatgaccgtcgcgcggccgagcgtgcccgcggcgctgcccctcctcggggagctgccccggctgctgctgctggtgctgttgtgcctgccggccgtgtggggtgactgtggccttcccccagatgtacctaatgcccagccagctttggaaggccgtacaagttttcccgaggatactgtaataacgtacaaatgtgaagaaagctttgtgaaaattcctggcgagaaggactcagtgatctgccttaagggcagtcaatggtcagatattgaagagttctgcaatcgtagctgcgaggtgccaacaaggctaaattctgcatccctcaaacagccttatatcactcagaattattttccagtcggtactgttgtggaatatgagtgccgtccaggttacagaagagaaccttctctatcaccaaaactaacttgccttcagaatttaaaatggtccacagcagtcgaattttgtaaaaagaaatcatgccctaatccgggagaaatacgaaatggtcagattgatgtaccaggtggcatattatttggtgcaaccatctccttctcatgtaacacagggtacaaattatttggctcgacttctagtttttgtcttatttcaggcagctctgtccagtggagtgacccgttgccagagtgcagagaaatttattgtccagcaccaccacaaattgacaatggaataattcaaggggaacgtgaccattatggatatagacagtctgtaacgtatgcatgtaataaaggattcaccatgattggagagcactctatttattgtactgtgaataatgatgaaggagagtggagtggcccaccacctgaatgcagaggaaaatctctaacttccaaggtcccaccaacagttcagaaacctaccacagtaaatgttccaactacagaagtctcaccaacttctcagaaaaccaccacaaaaaccaccacaccaaatgctcaagcaacacggagtacacctgtttccaggacaaccaagcattttcatgaaacaaccccaaataaaggaagtggaaccacttcaggtactacccgtcttctatctgggcacacgtgtttcacgttgacaggtttgcttgggacgctagtaaccatgggcttgctgacttaggcctcgactgtgccttctagttgccagccatctgttgtttgcccctcccccgtgccttccttgaccctggaaggtgccactcccactgtcctttcctaataaaatgaggaaattgcatcgcattgtctgagtaggtgtcattctattctggggggtggggtggggcaggacagcaagggggaggattgggaagacaatagcaggcatgctggggctagcgcggccgcggataacttcgtatagcatacattatacgaagttatgggattcttttgccctggcttaacctgattcttgggcgttgtcctgcaggggattgagcaggtgtacgaggacgagcccaatttctctatattcccacagtcttgagtttgtgtcacaaaataattatagtggggtggagatgggaaatgagtccaggcaacacctaagcctgattttatgcattgagactgcgtgttattactaaagatctttgtgtcgcaatttcctgatgaagggagataggttaaaaagcacggatctactgagttttacagtcatcccatttgtagacttttgctacaccaccaaagtatagcatctgagattaaatattaatctccaaaccttaggccccctcacttgcatccttacggtcagataactctcactcatactttaagcccattttgtttgttgtacttgctcatccagtcccagtcccattggctttctcctcacctgttttaggtagccagcaagtcatgaaatcagataagttccaccaccaattaacactacccatcttgagcataggcccaacagtgcatttattcctcatttactgatgttcgtgaatatttaccttgattttcatttttttctttttcttaagctgggattttactcctgaccctattcacagtcagatgatcttgactaccactgcgattggacctgaggttcagcaatactcccctttatgtcttttgaatacttttcaataaatctgtttgtattttcattagttagtaactgagctcagttgccgtaatgctaatagcttccaaactagtgtctctgtctccagtatctgataaatcttaggtgttgctgggacagttgtcctaaaattaagataaagcatgaaaataactgacacaactccattactggctcctaactacttaaacaatgcattctatcatcacaaatgtgaaaaaggagttccctcagtggactaaccttatcttttctcaacacctttttctttgcacaattttccacacatgcctacaaaaagtacttctctgctcaagtcacactgagttgattgctatttaccgaaatcaaagtaacattatcagatctctgtagggtggttccctctggaatgctaccctccatagtccttacccttcaagtaaagagcatgaagactgaaatatctctgtgatctgtcatcctttaagccagaatcccccataaaaaagttagtattgctttctcctgatcccatagcaggttgaatcatagcacttatcaggttgttgtcattgcttgcttaaattctcctaactatttggagcttcttgagggcacaggttcttgttgagtcttgtacctaagcacctagtatagtccttgatgtctagccaaccctaaataaaatgcagtgagtgacatgtagatgtctttataaggtttgataggttggtctctcaaacagttcttttgtatgtttggtagtgctctagattagcactggccagtataactctgatgatggaaatgttctatagctatgctgtctaatatggta

SEQ ID NO: 7 - RNA, 20 nt, synthetic construct
  source 1..20: mol_type = other RNA
gaggccattctctgatggac

SEQ ID NO: 8 - RNA, 20 nt, synthetic construct
  source 1..20: mol_type = other RNA
gtgactatattttgactaaa

SEQ ID NO: 9 - RNA, 20 nt, synthetic construct
  source 1..20: mol_type = other RNA
gagcatggtctgtctcttcc

SEQ ID NO: 10 - RNA, 21 nt, synthetic construct
  source 1..21: mol_type = other RNA
gtacttcattagtcccctaag

SEQ ID NO: 11 - DNA, 4096 bp, synthetic construct
  source 1..4096: mol_type = other DNA
agcttggcgtaatcatggtcatagctgtttcctgtgtgaaattgttatccgctcacaattccacacaacatacgagccggaagcataaagtgtaaagcctggggtgcctaatgagtgagctaactcacattaattgcgttgcgctcactgcccgctttccagtcgggaaacctgtcgtgccagctgcattaatgaatcggccaacgcgcggggagaggcggtttgcgtattgggcgctcttccgcttcctcgctcactgactcgctgcgctcggtcgttcggctgcggcgagcggtatcagctcactcaaaggcggtaatacggttatccacagaatcaggggataacgcaggaaagaacatgtgagcaaaaggccagcaaaaggccaggaaccgtaaaaaggccgcgttgctggcgtttttccataggctccgcccccctgacgagcatcacaaaaatcgacgctcaagtcagaggtggcgaaacccgacaggactataaagataccaggcgtttccccctggaagctccctcgtgcgctctcctgttccgaccctgccgcttaccggatacctgtccgcctttctcccttcgggaagcgtggcgctttctcatagctcacgctgtaggtatctcagttcggtgtaggtcgttcgctccaagctgggctgtgtgcacgaaccccccgttcagcccgaccgctgcgccttatccggtaactatcgtcttgagtccaacccggtaagacacgacttatcgccactggcagcagccactggtaacaggattagcagagcgaggtatgtaggcggtgctacagagttcttgaagtggtggcctaactacggctacactagaagaacagtatttggtatctgcgctctgctgaagccagttaccttcggaaaaagagttggtagctcttgatccggcaaacaaaccaccgctggtagcggtggtttttttgtttgcaagcagcagattacgcgcagaaaaaaaggatctcaagaagatcctttgatcttttctacggggtctgacgctcagtggaacgaaaactcacgttaagggattttggtcatgagattatcaaaaaggatcttcacctagatccttttaaattaaaaatgaagttttaaatcaatctaaagtatatatgagtaaacttggtctgacagttaccaatgcttaatcagtgaggcacctatctcagcgatctgtctatttcgttcatccatagttgcctgactccccgtcgtgtagataactacgatacgggagggcttaccatctggccccagtgctgcaatgataccgcgagacccacgctcaccggctccagatttatcagcaataaaccagccagccggaagggccgagcgcagaagtggtcctgcaactttatccgcctccatccagtctattaattgttgccgggaagctagagtaagtagttcgccagttaatagtttgcgcaacgttgttgccattgctacaggcatcgtggtgtcacgctcgtcgtttggtatggcttcattcagctccggttcccaacgatcaaggcgagttacatgatcccccatgttgtgcaaaaaagcggttagctccttcggtcctccgatcgttgtcagaagtaagttggccgcagtgttatcactcatggttatggcagcactgcataattctcttactgtcatgccatccgtaagatgcttttctgtgactggtgagtactcaaccaagtcattctgagaatagtgtatgcggcgaccgagttgctcttgcccggcgtcaatacgggataataccgcgccacatagcagaactttaaaagtgctcatcattggaaaacgttcttcggggcgaaaactctcaaggatcttaccgctgttgagatccagttcgatgtaacccactcgtgcacccaactgatcttcagcatcttttactttcaccagcgtttctgggtgagcaaaaacaggaaggcaaaatgccgcaaaaaagggaataagggcgacacggaaatgttgaatactcatactcttcctcccaagcttagctatggccgtttcttgagccttaataaagaccccaatgggatagttcaggctgggctgaccctataggtaggtagttgtatggttaataccagattgcagcgcgcaatttctaaaattaaacccacttagtaaacagtctgtttactgggtaatcatgtatatgatagtttctcccaaacaaatacccacgtttattgggacaaaagttgttagggaaaatggggcctcagagttatgattcaagtcataattctttccatttataatttcactcgagactctgttaactgattccttgtgtgttgtatcttactcctcagctcacaattacttttagttattcaccttaactgtatgaataacagtggagaaaaggattctaccagaatactctaattatggttttgagtcccctttccagactgaagatttttcagtctttttgatctgaggtgatttttcagtcttttcgatctgaggtgacagtctcaagctcctcaattcacccagtctcttgatacttgtccatttagggccaccaaagctactttgacttcatactagagagtcaattaatgaggccattctctgatggacaggtgaagcaggcaaggtgactatattttgactaaacggtagaaaacagcctgagtgttaacagtgtagcctataaaacccagagctgcccaccctgatctaaacttccaggaacataagaaagtaggtcacatttcagtaaaacctggctttgtggattgagcatggtctgtctcttcctggtacttcattagtcccctaagtgggatttgctgagcaagactggctccggtgcccgtcagtgggcagagcgcacatcgcccacagtccccgagaagttggggggaggggtcggcaattgaaccggtgcctagagaaggtggcgcggggtaaactgggaaagtgatgtcgtgtactggctccgcctttttcccgagggtgggggagaaccgtatataagtgcagtagtcgccgtgaacgttctttttcgcaacgggtttgccgccagaacacaggtaagtgccgtgtgtggttcccgcgggcctggcctctttacgggttatggcccttgcgtgccttgaattacttccacctggctgcagtacgtgattcttgatcccgagcttcgggttggaagtgggtgggagagttcgaggccttgcgcttaaggagccccttcgcctcgtgcttgagttgaggcctggcctgggcgctggggccgccgcgtgcgaatctggtggcaccttcgcgcctgtctcgctgctttcgataagtctctagccatttaaaatttttgatgacctgctgcgacgctttttttctggcaagatagtcttgtaaatgcgggccaagatctgcacactggtatttcggtttttggggccgcgggcggcgacggggcccgtgcgtcccagcgcacatgttcggcgaggcggggcctgcgagcgcggccaccgagaatcggacgggggtagtctcaagctggccggcctgctctggtgcctggcctcgcgccgccgtgtatcgccccgccctgggcggcaaggctggcccggtcggcaccagttgcgtgagcggaaagatggccgcttcccggccctgctgcagggagctcaaaatggaggacgcggcgctcgggagagcgggcgggtgagtcacccacacaaaggaaaagggcctttccgtcctcagccgtcgcttcatgtgactccacggagtaccgggcgccgtccaggcacctcgattagttctcgagcttttggagtacgtcgtctttaggttggggggaggggttttatgcgatggagtttccccacactgagtgggtggagactgaagttaggccagcttggcacttgatgtaattctccttggaatttgccctttttgagtttggatcttggttcattctcaagcctcagacagtggttcaaagtttttttcttccatttcaggtgtcgtgaaccatgtggcccctggtagcggcgctgttgctgggc